European Patent Specification EP 3 669 002 B1, published January 15, 2025. Title: MCC as epigenetic marker for the identification of immune cells, in particular basophil granulocytes. Applicant: Epiontis GmbH. The sequence listing filed with the application follows.

SEQUENCE LISTING (11 sequences)

SEQ ID NO: 1 - DNA, 406 bp, Homo sapiens
tgctctggtcctccttgcccaagaggtgtggggatgggtgtggtggaggcacagtccggggttggtctcgcctgccgcacgcctgttcagtagccttttaatgaactcagtgactcagcgctgtccctcccccaccggcctcggatctcattcctctcaatcgcactgatgcccatgtgacagcacgttgtctccaccgagactaatcccttatcaataagagctttcagcacggcccagaccagattactctgtctcacaaccactttgctgacctgcccggggggccaccgaatactccccgagcgcatactatttacagaagagtcaagataagccggatcacttggcgtgattatttcgcttccaaagtttgtggctttaacaaagcaaacccacattcaac

SEQ ID NO: 2 - DNA, 406 bp, Homo sapiens
tactctaatcctccttacccaaaaaatataaaaataaatataataaaaacacaatccaaaattaatctcacctaccacacacctattcaataaccttttaataaactcaataactcaacactatccctcccccaccaacctcaaatctcattcctctcaatcacactaatacccatataacaacacattatctccaccaaaactaatcccttatcaataaaaactttcaacacaacccaaaccaaattactctatctcacaaccactttactaacctacccaaaaaaccaccaaatactccccaaacacatactatttacaaaaaaatcaaaataaaccaaatcacttaacataattatttcacttccaaaatttataactttaacaaaacaaacccacattcaac

SEQ ID NO: 3 - DNA, 406 bp, Homo sapiens
tactctaatcctccttacccaaaaaatataaaaataaatataataaaaacacaatccgaaattaatctcgcctaccgcacgcctattcaataaccttttaataaactcaataactcaacgctatccctcccccaccgacctcgaatctcattcctctcaatcgcactaatacccatataacaacacgttatctccaccgaaactaatcccttatcaataaaaactttcaacacgacccaaaccaaattactctatctcacaaccactttactaacctacccgaaaaaccaccgaatactccccgaacgcatactatttacaaaaaaatcaaaataaaccgaatcacttaacgtaattatttcgcttccaaaatttataactttaacaaaacaaacccacattcaac

SEQ ID NO: 4 - DNA, 22 bp, Homo sapiens
tactctaatcctccttacccaa

SEQ ID NO: 5 - DNA, 20 bp, Homo sapiens
gttgaatgtgggtttgtttt

SEQ ID NO: 6 - DNA, 23 bp, Homo sapiens
aacacaatccaaaattaatctca

SEQ ID NO: 7 - DNA, 21 bp, Homo sapiens
gaggaatgagatttgaggttg

SEQ ID NO: 8 - DNA, 24 bp, Homo sapiens
attgaataggcgtgcggtaggcga

SEQ ID NO: 9 - DNA, 24 bp, Homo sapiens
aacacaatccgaaattaatctcgc

SEQ ID NO: 10 - DNA, 19 bp, Homo sapiens
ggaatgagattcgaggtcg

SEQ ID NO: 11 - DNA, 30 bp, Homo sapiens
aggttattgaataggtgtgtggtaggtgag